European Patent Specification EP 4 015 655 B1, published June 5, 2024. Title: COMPOSITION, KIT AND METHOD FOR DETECTING AND CLASSIFYING PATHOGENS CAUSING RESPIRATORY TRACT INFECTION, AND APPLICATION. Applicant: SANSURE BIOTECH INC. The sequence listing filed with the application follows.

SEQUENCE LISTING (28 sequences)

SEQ ID NO: 1 - DNA, 20 bp, Artificial sequence
cagaagatttgtccttccag

SEQ ID NO: 2 - DNA, 23 bp, Artificial sequence
gtcatactcctctgcattgtctc

SEQ ID NO: 3 - DNA, 27 bp, Artificial sequence
tcttcgagctctcggacgaaaaggcaa

SEQ ID NO: 4 - DNA, 19 bp, Artificial sequence
gccatcggatcctcaattc

SEQ ID NO: 5 - DNA, 22 bp, Artificial sequence
ttcttccgtgaccagtctaatt

SEQ ID NO: 6 - DNA, 27 bp, Artificial sequence
aaggacatccaaagccaattcgagcag

SEQ ID NO: 7 - DNA, 24 bp, Artificial sequence
caccctgacaaaatcaacaatata

SEQ ID NO: 8 - DNA, 22 bp, Artificial sequence
cataggcacccatattgttagt

SEQ ID NO: 9 - DNA, 26 bp, Artificial sequence
agacaagatggggcaaatatggaaac

SEQ ID NO: 10 - DNA, 22 bp, Artificial sequence
gcagtggtcttacatgcacatc

SEQ ID NO: 11 - DNA, 20 bp, Artificial sequence
tatcctcacggtccacaggg

SEQ ID NO: 12 - DNA, 25 bp, Artificial sequence
ccaggacgcctcggagtacctgagc

SEQ ID NO: 13 - DNA, 26 bp, Artificial sequence
agcaatctttaatcagtgtgtaacat

SEQ ID NO: 14 - DNA, 24 bp, Artificial sequence
aaatcacatggggatagcactact

SEQ ID NO: 15 - DNA, 26 bp, Artificial sequence
aaagagccaccacattttcaccgagg

SEQ ID NO: 16 - DNA, 20 bp, Artificial sequence
ctttggttcgcatgaatcaa

SEQ ID NO: 17 - DNA, 18 bp, Artificial sequence
ttccctactgctgcctcc

SEQ ID NO: 18 - DNA, 28 bp, Artificial sequence
tcgttatttgatgagggtgcgccatatc

SEQ ID NO: 19 - DNA, 21 bp, Artificial sequence
ctcctctgacttcaacagcga

SEQ ID NO: 20 - DNA, 18 bp, Artificial sequence
ccaccaccctgttgctgt

SEQ ID NO: 21 - DNA, 20 bp, Artificial sequence
ttgacgctggggctggcatt

SEQ ID NO: 22 - DNA, 132 bp, Homo sapiens
tctcctctgacttcaacagcgacacccactcctccacctttgacgctggggctggcattgccctcaacgaccactttgtcaagctcatttcctggtatgacaacgaatttggctacagcaacagggtggtgg

SEQ ID NO: 23 - DNA, 20 bp, Artificial sequence
gcggatgccttttgttgatt

SEQ ID NO: 24 - DNA, 21 bp, Artificial sequence
ttgcttcaaatgagaatgtgg

SEQ ID NO: 25 - DNA, 25 bp, Artificial sequence
ccactcctggtccttatggcccagt

SEQ ID NO: 26 - DNA, 25 bp, Artificial sequence
cactgatgacaatgcgttagcttac

SEQ ID NO: 27 - DNA, 29 bp, Artificial sequence
ccagttctgtatagatagtaccagttcca

SEQ ID NO: 28 - DNA, 29 bp, Artificial sequence
cggataacagtgcaagtacaaacctacct